European Patent Application EP 4 640 695 A1, published October 29, 2025. Title: 一种重组脊髓灰质炎病毒样颗粒及其制备方法和用途. Applicant: 康希诺生物股份公司. The sequence listing filed with the application follows.

SEQUENCE LISTING (16 sequences)

SEQ ID NO: 1 - protein, 22 aa, synthetic construct
GSGATNFSLLKQAGDVEENPGP

SEQ ID NO: 2 - protein, 881 aa, synthetic construct
MGAQVSSQKVGAHENSNRAYGGSTINYTTINYYRDSASNAASKQDFSQDPSKFTEPIKDVLIKTSPMLNSPNIEACGYSDRVLQLTLGNSTITTQEAANSVVAYGRWPEYLRDSEANPVDQPTEPDVAACRFYTLDTVSWTKESRGWWWKLPDALRDMGLFGQNMYYHYLGRSGYTVHVQCNASKFHQGALGVFAVPEMCLAGDSNTTTMHTSYQNANPGEKGGTFTGTFTPDDNQTSPARRFCPVDYLFGNGTLLGNAFVFPHQIINLRTNNCATLVLPYVNSLSIDSMVKHNNWGIAILPLAPLNFASESSPEIPITLTIAPMCCEFNGLRNITLPRLQGLPVMNTPGSNQYLTADNFQSPCALPEFDVTPPIDIPGEVKNMMELAEIDTMIPFDLSAKKKNTMEMYRVRLSDKPHTDDPILCLSLSPASDPRLSHTMLGEILNYYTHWAGSLKFTFLFCGSMMATGKLLVSYAPPGADPPKKRKEAMLGTHVIWDIGLQSSCTMVVPWISNTTYRQTIDDSFTEGGYISVFYQTRIVVPLSTPREMDILGFVSACNDFSVRLMRDTTHIEQKALAQGLGQMLESMIDNTVRETVGAATSRDALPNTEASGPAHSKEIPALTAVETGATNPLVPSDTVQTRHVVQHRSRSESSIESFFARGACVAIITVDNSASTKNKDKLFTVWKITYKDTVQLRRKLEFFTYSRFDMEFTFVVTANFTETNNGHALNQVYQIMYVPPGAPVPEKWDDYTWQTSSNPSIFYTYGTAPARISVPYVGISNAYSHFYDGFSKVPLKDQSAALGDSLYGAASLNDFGILAVRVVNDHNPTKVTSKIRVYLKPKHIRVWCPRPPRAVAYYGPGVDYKDGTLTPLSTKDLTTY

SEQ ID NO: 3 - protein, 302 aa, synthetic construct
GLGQMLESMIDNTVRETVGAATSRDALPNTEASGPAHSKEIPALTAVETGATNPLVPSDTVQTRHVVQHRSRSESSIESFFARGACVAIITVDNSASTKNKDKLFTVWKITYKDTVQLRRKLEFFTYSRFDMEFTFVVTANFTETNNGHALNQVYQIMYVPPGAPVPEKWDDYTWQTSSNPSIFYTYGTAPARISVPYVGISNAYSHFYDGFSKVPLKDQSAALGDSLYGAASLNDFGILAVRVVNDHNPTKVTSKIRVYLKPKHIRVWCPRPPRAVAYYGPGVDYKDGTLTPLSTKDLTTY

SEQ ID NO: 4 - protein, 341 aa, synthetic construct
MGAQVSSQKVGAHENSNRAYGGSTINYTTINYYRDSASNAASKQDFSQDPSKFTEPIKDVLIKTSPMLNSPNIEACGYSDRVLQLTLGNSTITTQEAANSVVAYGRWPEYLRDSEANPVDQPTEPDVAACRFYTLDTVSWTKESRGWWWKLPDALRDMGLFGQNMYYHYLGRSGYTVHVQCNASKFHQGALGVFAVPEMCLAGDSNTTTMHTSYQNANPGEKGGTFTGTFTPDDNQTSPARRFCPVDYLFGNGTLLGNAFVFPHQIINLRTNNCATLVLPYVNSLSIDSMVKHNNWGIAILPLAPLNFASESSPEIPITLTIAPMCCEFNGLRNITLPRLQ

SEQ ID NO: 5 - protein, 238 aa, synthetic construct
GLPVMNTPGSNQYLTADNFQSPCALPEFDVTPPIDIPGEVKNMMELAEIDTMIPFDLSAKKKNTMEMYRVRLSDKPHTDDPILCLSLSPASDPRLSHTMLGEILNYYTHWAGSLKFTFLFCGSMMATGKLLVSYAPPGADPPKKRKEAMLGTHVIWDIGLQSSCTMVVPWISNTTYRQTIDDSFTEGGYISVFYQTRIVVPLSTPREMDILGFVSACNDFSVRLMRDTTHIEQKALAQ

SEQ ID NO: 6 - protein, 272 aa, synthetic construct
SPNIEACGYSDRVLQLTLGNSTITTQEAANSVVAYGRWPEYLRDSEANPVDQPTEPDVAACRFYTLDTVSWTKESRGWWWKLPDALRDMGLFGQNMYYHYLGRSGYTVHVQCNASKFHQGALGVFAVPEMCLAGDSNTTTMHTSYQNANPGEKGGTFTGTFTPDDNQTSPARRFCPVDYLFGNGTLLGNAFVFPHQIINLRTNNCATLVLPYVNSLSIDSMVKHNNWGIAILPLAPLNFASESSPEIPITLTIAPMCCEFNGLRNITLPRLQ

SEQ ID NO: 7 - protein, 879 aa, synthetic construct
MGAQVSSQKVGAHENSNRAYGGSTINYTTINYYRDSASNAASKQDFAQDPSKFTEPIKDVLIKTAPTLNSPNIEACGYSDRVMQLTLGNSTITTQEAANSVVAYGRWPEYIKDSEANPVDQPTEPDVAACRFYTLDTVTWRKESRGWWWKLPDALKDMGLFGQNMFYHYLGRAGYTVHVQCNASKFHQGALGVFAVPEMCLAGDSTTHMFTKYENANPGEKGGEFKGSFTLDTNATNPARNFCPVDYLFGSGVLAGNAFVYPHQIINLRTNNCATLVLPYVNSLSIDSMTKHNNWGIAILPLAPLDFATESSTEIPITLTIAPMCCEFNGLRNITVPRTQGLPVLNTPGSNQYLTADNYQSPCAIPEFDVTPPIDIPGEVRNMMELAEIDTMIPLNLTNQRKNTMDMYRVELNDAAHSDTPILCLSLSPASDPRLAHTMLGEILNYYTHWAGSLKFTFLFCGSMMATGKLLVSYAPPGAEAPKSRKEAMLGTHVIWDIGLQSSCTMVVPWISNTTYRQTINDSFTEGGYISMFYQTRVVVPLSTPRKMDILGFVSACNDFSVRLLRDTTHISQEAMPQGLGDLIEGVVEGVTRNALTPLTPANNLPDTQSSGPAHSKETPALTAVETGATNPLVPSDTVQTRHVIQKRTRSESTVESFFARGACVAIIEVDNDAPTKRASKLFSVWKITYKDTVQLRRKLEFFTYSRFDMEFTFVVTSNYTDANNGHALNQVYQIMYIPPGAPIPGKWNDYTWQTSSNPSVFYTYGAPPARISVPYVGIANAYSHFYDGFAKVPLAGQASTEGDSLYGAASLNDFGSLAVRVVNDHNPTKLTSKIRVYMKPKHVRVWCPRPPRAVPYYGPGVDYKDGLAPLPEKGLTTY

SEQ ID NO: 8 - protein, 301 aa, synthetic construct
GLGDLIEGVVEGVTRNALTPLTPANNLPDTQSSGPAHSKETPALTAVETGATNPLVPSDTVQTRHVIQKRTRSESTVESFFARGACVAIIEVDNDAPTKRASKLFSVWKITYKDTVQLRRKLEFFTYSRFDMEFTFVVTSNYTDANNGHALNQVYQIMYIPPGAPIPGKWNDYTWQTSSNPSVFYTYGAPPARISVPYVGIANAYSHFYDGFAKVPLAGQASTEGDSLYGAASLNDFGSLAVRVVNDHNPTKLTSKIRVYMKPKHVRVWCPRPPRAVPYYGPGVDYKDGLAPLPEKGLTTY

SEQ ID NO: 9 - protein, 340 aa, synthetic construct
MGAQVSSQKVGAHENSNRAYGGSTINYTTINYYRDSASNAASKQDFAQDPSKFTEPIKDVLIKTAPTLNSPNIEACGYSDRVMQLTLGNSTITTQEAANSVVAYGRWPEYIKDSEANPVDQPTEPDVAACRFYTLDTVTWRKESRGWWWKLPDALKDMGLFGQNMFYHYLGRAGYTVHVQCNASKFHQGALGVFAVPEMCLAGDSTTHMFTKYENANPGEKGGEFKGSFTLDTNATNPARNFCPVDYLFGSGVLAGNAFVYPHQIINLRTNNCATLVLPYVNSLSIDSMTKHNNWGIAILPLAPLDFATESSTEIPITLTIAPMCCEFNGLRNITVPRTQ

SEQ ID NO: 10 - protein, 238 aa, synthetic construct
GLPVLNTPGSNQYLTADNYQSPCAIPEFDVTPPIDIPGEVRNMMELAEIDTMIPLNLTNQRKNTMDMYRVELNDAAHSDTPILCLSLSPASDPRLAHTMLGEILNYYTHWAGSLKFTFLFCGSMMATGKLLVSYAPPGAEAPKSRKEAMLGTHVIWDIGLQSSCTMVVPWISNTTYRQTINDSFTEGGYISMFYQTRVVVPLSTPRKMDILGFVSACNDFSVRLLRDTTHISQEAMPQ

SEQ ID NO: 11 - protein, 271 aa, synthetic construct
SPNIEACGYSDRVMQLTLGNSTITTQEAANSVVAYGRWPEYIKDSEANPVDQPTEPDVAACRFYTLDTVTWRKESRGWWWKLPDALKDMGLFGQNMFYHYLGRAGYTVHVQCNASKFHQGALGVFAVPEMCLAGDSTTHMFTKYENANPGEKGGEFKGSFTLDTNATNPARNFCPVDYLFGSGVLAGNAFVYPHQIINLRTNNCATLVLPYVNSLSIDSMTKHNNWGIAILPLAPLDFATESSTEIPITLTIAPMCCEFNGLRNITVPRTQ

SEQ ID NO: 12 - protein, 878 aa, synthetic construct
MGAQVSSQKVGAHENSNRAYGGSTINYTTINYYKDSASNAASKQDYSQDPSKFTEPLKDVLIKTAPALNSPNVEACGYSDRVLQLTLGNSTITTQEAANSVVAYGRWPEFIRDDEANPVDQPTEPDVATCRFYTLDTVMWGKESKGWWWKLPDALRDMGLFGQNMYYHYLGRSGYTVHVQCNASKFHQGALGVFAIPEYCLAGDSDKQRYTSYANANPGERGGKFYSQFNKDNAVTSPKREFCPVDYLLGCGVLLGNAFVYPHQIINLRTNNSATIVLPYVNALAIDSMVKHNNWGIAILPLSPLDFAQDSSVEIPITVTIAPMCSEFNGLRNVTAPKFQGLPVLNTPGSNQYLTSDNHQSPCAIPEFDVTPPIDIPGEVKNMMELAEIDTMIPLNLESTKRNTMDMYRVTLSDSADLSQPILCLSLSPAFDPRLSHTMLGEVLNYYTHWAGSLKFTFLFCGSMMATGKILVAYAPPGAQPPTSRKEAMLGTHVIWDLGLQSSCTMVVPWISNVTYRQTTQDSFTEGGYISMFYQTRIVVPLSTPKSMSMLGFVSACNDFSVRLLRDTTHISQSALPQGIEDLTSEVAQGALTLSLPKQQDSLPDTKASGPAHSKEVPALTAVETGATNPLAPSDTVQTRHVVQRRSRSESTIESFFARGACVAIIEVDNEQPTTRAQKLFAMWRITYKDTVQLRRKLEFFTYSRFDMEFTFVVTANFTNANNGHALNQVYQIMYIPPGAPTPKSWDDYTWQTSSNPSIFYTYGAAPARISVPYVGLANAYSHFYDGFAKVPLKTDANDQIGDSLYSAMTVDDFGVLAVRVVNDHNPTKVTSKVRIYMKPKHVRVWCPRPPRAVPYYGPGVDYRNNLDPLSEKGLTTY

SEQ ID NO: 13 - protein, 300 aa, synthetic construct
GIEDLTSEVAQGALTLSLPKQQDSLPDTKASGPAHSKEVPALTAVETGATNPLAPSDTVQTRHVVQRRSRSESTIESFFARGACVAIIEVDNEQPTTRAQKLFAMWRITYKDTVQLRRKLEFFTYSRFDMEFTFVVTANFTNANNGHALNQVYQIMYIPPGAPTPKSWDDYTWQTSSNPSIFYTYGAAPARISVPYVGLANAYSHFYDGFAKVPLKTDANDQIGDSLYSAMTVDDFGVLAVRVVNDHNPTKVTSKVRIYMKPKHVRVWCPRPPRAVPYYGPGVDYRNNLDPLSEKGLTTY

SEQ ID NO: 14 - protein, 340 aa, synthetic construct
MGAQVSSQKVGAHENSNRAYGGSTINYTTINYYKDSASNAASKQDYSQDPSKFTEPLKDVLIKTAPALNSPNVEACGYSDRVLQLTLGNSTITTQEAANSVVAYGRWPEFIRDDEANPVDQPTEPDVATCRFYTLDTVMWGKESKGWWWKLPDALRDMGLFGQNMYYHYLGRSGYTVHVQCNASKFHQGALGVFAIPEYCLAGDSDKQRYTSYANANPGERGGKFYSQFNKDNAVTSPKREFCPVDYLLGCGVLLGNAFVYPHQIINLRTNNSATIVLPYVNALAIDSMVKHNNWGIAILPLSPLDFAQDSSVEIPITVTIAPMCSEFNGLRNVTAPKFQ

SEQ ID NO: 15 - protein, 238 aa, synthetic construct
GLPVLNTPGSNQYLTSDNHQSPCAIPEFDVTPPIDIPGEVKNMMELAEIDTMIPLNLESTKRNTMDMYRVTLSDSADLSQPILCLSLSPAFDPRLSHTMLGEVLNYYTHWAGSLKFTFLFCGSMMATGKILVAYAPPGAQPPTSRKEAMLGTHVIWDLGLQSSCTMVVPWISNVTYRQTTQDSFTEGGYISMFYQTRIVVPLSTPKSMSMLGFVSACNDFSVRLLRDTTHISQSALPQ

SEQ ID NO: 16 - protein, 271 aa, synthetic construct
SPNVEACGYSDRVLQLTLGNSTITTQEAANSVVAYGRWPEFIRDDEANPVDQPTEPDVATCRFYTLDTVMWGKESKGWWWKLPDALRDMGLFGQNMYYHYLGRSGYTVHVQCNASKFHQGALGVFAIPEYCLAGDSDKQRYTSYANANPGERGGKFYSQFNKDNAVTSPKREFCPVDYLLGCGVLLGNAFVYPHQIINLRTNNSATIVLPYVNALAIDSMVKHNNWGIAILPLSPLDFAQDSSVEIPITVTIAPMCSEFNGLRNVTAPKFQ